European Patent Specification EP 3 500 278 B1, published May 22, 2024. Title: METHODS AND COMPOSITIONS FOR TREATING CONDITIONS USING RECOMBINANT SELF-COMPLEMENTARY ADENO-ASSOCIATED VIRUS. Applicant: CALIMMUNE, INC. The sequence listing filed with the application follows.

SEQUENCE LISTING (7 sequences)

SEQ ID NO: 1 - DNA, 5718 bp, Artificial Sequence
  Sequence of Hu-IL-1Ra plasmid containing entire viral sequence with modified human IL1Ra insert and the SacII / NotI restriction sites.
cattaatgaatcggccaacgcgcggggagaggcggtttgcgtattgggcgctcttccgcttcctcgctcactgactcgctgcgctcggtcgttcggctgcggcgagcggtatcagctcactcaaaggcggtaatacggttatccacagaatcaggggataacgcaggaaagaacatgtgagcaaaaggccagcaaaaggccaggaaccgtaaaaaggccgcgttgctggcgtttttccataggctccgcccccctgacgagcatcacaaaaatcgacgctcaagtcagaggtggcgaaacccgacaggactataaagataccaggcgtttccccctggaagctccctcgtgcgctctcctgttccgaccctgccgcttaccggatacctgtccgcctttctcccttcgggaagcgtggcgctttctcatagctcacgctgtaggtatctcagttcggtgtaggtcgttcgctccaagctgggctgtgtgcacgaaccccccgttcagcccgaccgctgcgccttatccggtaactatcgtcttgagtccaacccggtaagacacgacttatcgccactggcagcagccactggtaacaggattagcagagcgaggtatgtaggcggtgctacagagttcttgaagtggtggcctaactacggctacactagaaggacagtatttggtatctgcgctctgctgaagccagttaccttcggaaaaagagttggtagctcttgatccggcaaacaaaccaccgctggtagcggtggtttttttgtttgcaagcagcagattacgcgcagaaaaaaaggatctcaagaagatcctttgatcttttctacggggtctgacgctcagtggaacgaaaactcacgttaagggattttggtcatgagattatcaaaaaggatcttcacctagatccttttaaattaaaaatgaagttttaaatcaatctaaagtatatatgagtaaacttggtctgacagttaccaatgcttaatcagtgaggcacctatctcagcgatctgtctatttcgttcatccatagttgcctgactccccgtcgtgtagataactacgatacgggagggcttaccatctggccccagtgctgcaatgataccgcgagacccacgctcaccggctccagatttatcagcaataaaccagccagccggaagggccgagcgcagaagtggtcctgcaactttatccgcctccatccagtctattaattgttgccgggaagctagagtaagtagttcgccagttaatagtttgcgcaacgttgttgccattgctacaggcatcgtggtgtcacgctcgtcgtttggtatggcttcattcagctccggttcccaacgatcaaggcgagttacatgatcccccatgttgtgcaaaaaagcggttagctccttcggtcctccgatcgttgtcagaagtaagttggccgcagtgttatcactcatggttatggcagcactgcataattctcttactgtcatgccatccgtaagatgcttttctgtgactggtgagtactcaaccaagtcattctgagaatagtgtatgcggcgaccgagttgctcttgcccggcgtcaatacgggataataccgcgccacatagcagaactttaaaagtgctcatcattggaaaacgttcttcggggcgaaaactctcaaggatcttaccgctgttgagatccagttcgatgtaacccactcgtgcacccaactgatcttcagcatcttttactttcaccagcgtttctgggtgagcaaaaacaggaaggcaaaatgccgcaaaaaagggaataagggcgacacggaaatgttgaatactcatactcttcctttttcaatattattgaagcatttatcagggttattgtctcatgagcggatacatatttgaatgtatttagaaaaataaacaaataggggttccgcgcacatttccccgaaaagtgccacctgacgtctaagaaaccattattatcatgacattaacctataaaaataggcgtatcacgaggccctttcgtctcgcgcgtttcggtgatgacggtgaaaacctctgacacatgcagctcccggagacggtcacagcttgtctgtaagcggatgccgggagcagacaagcccgtcagggcgcgtcagcgggtgttggcgggtgtcggggctggcttaactatgcggcatcagagcagattgtactgagagtgcaccatatgcggtgtgaaataccgcacagatgcgtaaggagaaaataccgcatcaggaattccaacatccaataaatcatacaggcaaggcaaagaattagcaaaattaagcaataaagcctcagagcataaagctaaatcggttgtaccaaaaacattatgaccctgtaatacttttgcgggagaagcctttatttcaacgcaaggataaaaatttttagaaccctcatatattttaaatgcaatgcctgagtaatgtgtaggtaaagattcaaacgggtgagaaaggccggagacagtcaaatcaccatcaatatgatattcaaccgttctagctgataaattcatgccggagagggtagctatttttgagaggtctctacaaaggctatcaggtcattgcctgagagtctggagcaaacaagagaatcgatgaacggtaatcgtaaaactagcatgtcaatcatatgtaccccggttgataatcagaaaagccccaaaaacaggaagattgtataagcaaatatttaaattgtaaacgttaatattttgttaaaattcgcgttaaatttttgttaaatcagctcattttttaaccaataggccgaaatcggcaaaatcccttataaatcaaaagaatagaccgagatagggttgagtgttgttccagtttggaacaagagtccactattaaagaacgtggactccaacgtcaaagggcgaaaaaccgtctatcagggcgatggcccactacgtgaaccatcaccctaatcaagttttttggggtcgaggtgccgtaaagcactaaatcggaaccctaaagggagcccccgatttagagcttgacggggaaagccggcgaacgtggcgagaaaggaagggaagaaagcgaaaggagcgggcgctagggcgctggcaagtgtagcggtcacgctgcgcgtaaccaccacacccgccgcgcttaatgcgccgctacagggcgcgtactatggttgctttgacgagcacgtataacgtgctttcctcgttagaatcagagcgggagctaaacaggaggccgattaaagggattttagacaggaacggtacgccagaatcctgagaagtgtttttataatcagtgaggccaccgagtaaaagagtctgtccatcacgcaaattaaccgttgtcgcaatacttctttgattagtaataacatcacttgcctgagtagaagaactcaaactatcggccttgctggtaatatccagaacaatattaccgccagccattgcaacaggaaaaacgctcatggaaatacctacattttgacgctcaatcgtctggaattccattcgccattcaggctgcgcaactgttgggaagggcgatcggtgcgggcctcttcgctattacgccagctggcgcgctcgctcgctcactgaggccgcccgggcaaagcccgggcgtcgggcgacctttggtcgcccggcctcagtgagcgagcgagcgcgcagagagggagtggccaactccatcactaggggttccttgtagttaatgattaacccgccatgctacttatctacgtagccatgctcgatctgaattcggtacccgttacataacttacggtaaatggcccgcctggctgaccgcccaacgacccccgcccattgacgtcaataatgacgtatgttcccatagtaacgccaatagggactttccattgacgtcaatgggtggagtatttacggtaaactgcccacttggcagtacatcaagtgtatcatatgccaagtacgccccctattgacgtcaatgacggtaaatggcccgcctggcattatgcccagtacatgaccttatgggactttcctacttggcagtacatctacgtattagtcatcgctattaccatggtgatgcggttttggcagtacatcaatgggcgtggatagcggtttgactcacggggatttccaagtctccaccccattgacgtcaatgggagtttgttttggcaccaaaatcaacgggactttccaaaatgtcgtaacaactccgccccattgacgcaaatgggcggtaggcgtgtacggtgggaggtctatataagcagagctcgtttagtgaaccgtcagatcgcctggagacgccatccacgctgttttgacctccatagaagacaccgggaccgatccagcctccggactctagaggatccggtactcgaggaactgaaaaaccagaaagttaactggtaagtttagtctttttgtcttttatttcaggtcccggatccggtggtggtgcaaatcaaagaactgctcctcagtggatgttgcctttacttctaggcctgtacggaagtgttacttctgctctaaaagctgcggaattgtacccgcgggccaccatggaaatctgcagaggcctgcggagccacctgattaccctgctgctgttcctgttccacagcgagacaatctgccggcccagcggccggaagtccagcaagatgcaggccttccggatctgggacgtgaaccagaaaaccttctacctgcggaacaaccagctggtggccggatacctgcagggccccaacgtgaacctggaagagaagatcgacgtggtgcccatcgagccccacgccctgtttctgggcatccacggcggcaagatgtgcctgagctgcgtgaagtccggcgacgagacaagactgcagctggaagccgtgaacatcaccgacctgagcgagaaccggaagcaggacaagagattcgccttcatcagaagcgacagcggccccaccaccagctttgagagcgccgcctgccccggctggttcctgtgtacagccatggaagccgaccagcccgtgtccctgacaaacatgcccgacgagggcgtgatggtcaccaagttctattttcaagaagatgagtaataagcggccgccgggatccagacatgataagatacattgatgagtttggacaaaccacaactagaatgcagtgaaaaaaatgctttatttgtgaaatttgtgatgctattgctttatttgtaaccattataagctgcaataaacaagttaacaacaacaattgcattcattttatgtttcaggttcagggggaggtgtgggaggttttttagtcgactagagctcgctgatcagcctcgactgtgccttctagttgccagccatctgttgtttgcccctcccccgtgccttccttgaccctggaaggtgccactcccactgtcctttcctaataaaatgaggaaattgcatcgcattgtctgagtaggtgtcattctattctggggggtggggtggggcaggacagcaagggggaggattgggaagacaatagcaggaaccccactccctctctgcgcgctcgctcgctcactgaggccgggcgaccaaaggtcgcccgacgcccgggctttgcccgggcggcctcagtgagcgagcgagcgcgcagctgctg

SEQ ID NO: 2 - DNA, 537 bp, Artificial Sequence
  Modified human IL-1Ra insert
atggaaatctgcagaggcctgcggagccacctgattaccctgctgctgttcctgttccacagcgagacaatctgccggcccagcggccggaagtccagcaagatgcaggccttccggatctgggacgtgaaccagaaaaccttctacctgcggaacaaccagctggtggccggatacctgcagggccccaacgtgaacctggaagagaagatcgacgtggtgcccatcgagccccacgccctgtttctgggcatccacggcggcaagatgtgcctgagctgcgtgaagtccggcgacgagacaagactgcagctggaagccgtgaacatcaccgacctgagcgagaaccggaagcaggacaagagattcgccttcatcagaagcgacagcggccccaccaccagctttgagagcgccgcctgccccggctggttcctgtgtacagccatggaagccgaccagcccgtgtccctgacaaacatgcccgacgagggcgtgatggtcaccaagttctattttcaagaagatgagtaataa

SEQ ID NO: 3 - DNA, 537 bp, Artificial Sequence
  Modified human IL-1Ra insert  (98% identical to SEQ ID NO: 2;
atggaaatctgcagaggactgcggagccacctaattaccctactccttttcctgttccacagcgagacaatctgccggcccagcggccggaagtccagcaagatgcaggctttccggatctgggacgtgaaccagaaaaccttctacctccggaacaaccagctggtggcgggatacctccagggccccaacgtgaacctagaagagaagatcgacgtggtgcccatcgagccccacgccctgtttctgggcatccacggcggcaagatgtgcctgagctgcgtgaagtccggcgacgagacaagactgcagctggaagccgtgaacatcaccgacctgagcgagaaccggaagcaggacaagagattcgccttcatcagaagcgacagcggccccaccaccagctttgagagcgccgcctgccccggctggttcctgtgtacagccatggaagccgaccagcccgtgtccctgacaaacatgcccgacgagggcgtgatggtcaccaagttctattttcaagaagatgagtaataa

SEQ ID NO: 4 - DNA, 537 bp, Artificial Sequence
  Modified human IL-1Ra insert  (99% identical to SEQ ID NO: 2;
atggagatctgcagaggcctgcggagccatctgattaccctactgcttttcctgttccatagcgagacaatctgccggcccagcggccggaagtccagcaaaatgcaggccttccggatctgggacgtgaaccagaaaaccttctacctgcggaacaaccagctggtggccggatacctgcagggccccaacgtgaacctggaagagaagatcgacgtggtgcccatcgagccccacgccctgtttctgggcatccacggcggcaagatgtgcctgagctgcgtgaagtccggcgacgagacaagactgcagctggaagccgtgaacatcaccgacctgagcgagaaccggaagcaggacaagagattcgccttcatcagaagcgacagcggccccaccaccagctttgagagcgccgcctgccccggctggttcctgtgtacagccatggaagccgaccagcccgtgtccctgacaaacatgcccgacgagggcgtgatggtcaccaagttctattttcaagaagatgagtaataa

SEQ ID NO: 5 - DNA, 537 bp, Artificial Sequence
  Modified human IL-1Ra insert  (95% identical to SEQ ID NO: 2;
atggagatctgcagaggactgcggagccacctaattaccctactccttttcctgttccatagcgagacaatctgccggcccagcggccggaagtccagcaaaatgcaggctttccggatctgggatgtgaaccagaagaccttctacctccggaacaaccagctggtggcgggatacctccagggccccaacgtgaacctagaagagaagatcgacgtggtgcccatcgagccccacgccctgtttctgggcatccatggcggcaagatgtgtctgagttgcgtgaagtcaggcgacgagacaagactgcagctggaagccgtgaacatcaccgacctgagcgaaaaccggaagcaggacaagagattcgccttcatcagaagcgacagcggccccaccactagctttgagagcgcagcctgccccggctggttcctgtgtacagccatggaggccgaccagcccgtgtccctgacaaacatgcctgacgaaggcgtgatggtcaccaagttctactttcaagaagatgaataataa

SEQ ID NO: 6 - protein, 177 aa, Homo sapiens
MEICRGLRSHLITLLLFLFHSETICRPSGRKSSKMQAFRIWDVNQKTFYLRNNQLVAGYLQGPNVNLEEKIDVVPIEPHALFLGIHGGKMCLSCVKSGDETRLQLEAVNITDLSENRKQDKRFAFIRSDSGPTTSFESAACPGWFLCTAMEADQPVSLTNMPDEGVMVTKFYFQEDE

SEQ ID NO: 7 - DNA, 1165 bp, Artificial Sequence
  IL-1 beta/ IL-6 hybrid promoter
atccaagagggagaagaagcccattggagatgatgccataaaggaagtggaagcgatatgataaaaatcatagtgcccattcccaaataatcccagaagcagaagggaaaggagagaaatatccacaaagacaggtgtgggtacacacaacatttttcatactttaagatcccagaggactcatggaaatgatacaagaaaatgactcataagaacaaatattaggaagccagtgccaagaatgagatgggaaattggggaaaatgttgggggcagattgcttagttctgttctaagcaagagggtgaacaaggaaggaacagctcactacaaagaacagacatcactgcatgtacacacaataatataagaactaacccatgattattttgcttgtcttcttgttcaaaatgattgaagaccaatgagatgagatcaaccttgataactggctggcttcggcatgattagacacaagatggtatcagggcacttgctgctttgaataatgtcagtctcctgtcttggaagaatgacctgacagggtaaagaggaacttgcagctgagaaaggctttagtgactcaagagctgaataattccccaaaagctggagcatcctggcatttccagctccccatctctgcttgttccacttccttggggctacatcaccatctacatcatcatcactcttccactccctcccttagtgccaactatgtttatagcgagatattttctgctcattggggatcggaaggaagtgctgtggcctgagcggtctccttgggaagacaggatctgatacatacgttgcacaacctatttgacataagaggtttcacttcctgagatggatgggatggtagcagatttgggtccaggttacagggccaggatgagacatggcagaactgtggagactgttacgtcagggggcattgccccatggctccaaaatttccctcgagcctctggccccaccctcaccctccaacaaagatttatcaaatgtgggattttcccatgagtctcaatattagagtctcaacccccaataaatataggactggagatgtctgaggctcattctgccctcgagcccaccgggaacgaaagagaagctctatctcccctccaggagcccagctatgaactccttc